European Patent Specification EP 3 907 232 B1, published February 21, 2024. Title: IMPROVED VACCINES AND METHODS FOR USING THE SAME. Applicant: The Trustees of the University of Pennsylvania. The sequence listing filed with the application follows.

SEQUENCE LISTING (43 sequences)

SEQ ID NO: 1 - DNA, 2142 bp, Artificial Sequence
  Subtype A consensus Envelope DNA sequence construct
ggatccatggactggacctggattctgttcctggtggccgccgccaccagagtgcacagcagagtgatgggcatccagcggaattgccagcacctgtggagatggggcaccatgatcctgggcatgatcatcatctgctctgccgccgagaacctgtgggtgaccgtgtactacggcgtgcctgtgtggaaggacgccgagaccaccctgttctgcgccagcgacgccaaggcctacgataccgaagtgcacaatgtgtgggccacccacgcctgcgtgcctaccgatcccaacccccaggagatcaacctggagaacgtgaccgaggagttcaacatgtggaagaacaacatggtggagcagatgcacaccgacatcatcagcctgtgggaccagagcctgaagccttgcgtgaagctgacccctctgtgcgtgaccctgaactgcagcaacgtgaacgtgaccaccaacatcatgaagggcgagatcaagaactgcagcttcaacatgaccaccgagctgcgggacaagaagcagaaagtgtacagcctgttctacaagctggacgtggtgcagatcaacaagagcaacagcagcagccagtaccggctgatcaactgcaacaccagcgccatcacccaggcctgccccaaagtgagcttcgagcccatccccatccactactgcgcccctgccggcttcgccatcctgaagtgcaaggacaaggagtttaacggcaccggcccctgcaagaatgtgagcaccgtgcagtgcacccacggcatcaagcccgtggtgtccacccagctgctgctgaacggcagcctggccgaggaggaagtgatgatccggagcgagaacatcaccaacaacgccaagaacatcatcgtgcagctgaccaagcccgtgaagatcaattgcacccggcccaacaacaacacccggaagagcatcagaatcggccctggccaggccttctacgccaccggcgacatcatcggcgatatcaggcaggcccactgcaatgtgagccggaccgagtggaacgagaccctgcagaaagtggccaagcagctgcggaagtacttcaacaacaagaccatcatcttcaccaacagcagcggcggcagactgagaatcaccacccacagcttcaattgtggcggcgagttcttctactgcaatacctccggcctgttcaacagcacctggaacggcaacggcaccaagaagaagaacagcaccgagagcaacgacaccatcaccctgccctgccggatcaagcagatcatcaatatgtggcagagggtgggccaggccatgtacgcccctcccatccagggcgtgatcagatgcgagagcaacatcaccggcctgctgctgaccagagatggcggcgacaacaacagcaagaacgagaccttcagacctggcggcggagacatgagggacaactggcggagcgagctgtacaagtacaaagtggtgaagatcgagcccctgggcgtggcccccaccaaggccaagagaagagtggtggagcgggagaagagagctgtgggcatcggcgccgtgttcctgggcttcctgggagccgccggaagcaccatgggagccgccagcatcaccctgaccgtgcaggccagacagctgctgagcggcattgtgcagcagcagagcaacctgctgagagccatcgaggcccagcagcacctgctgaagctgacagtgtggggcatcaaacagctgcaggcccgcgtgctggccgtggagagatacctgaaggaccagcagctgctgggcatctggggctgcagcggcaagctgatctgcaccaccaacgtgccctggaatagcagctggagcaacaagagccagagcgagatctgggacaacatgacctggctgcagtgggacaaggagatcagcaactacaccgatatcatctacaacctgatcgaggagagccagaaccagcaggagaagaacgagcaggatctgctggccctggacaagtgggccaacctgtggaactggttcgacatcagcaactggctgtggtacatcaagatcttcatcatgattgtgggcggcctgatcggcctgagaatcgtgttcgccgtgctgtctgtgtgactcgag

SEQ ID NO: 2 - protein, 709 aa, Artificial Sequence
  Subtype A consensus Envelope protein sequence construct
MDWTWILFLVAAATRVHSRVMGIQRNCQHLWRWGTMILGMIIICSAAENLWVTVYYGVPVWKDAETTLFCASDAKAYDTEVHNVWATHACVPTDPNPQEINLENVTEEFNMWKNNMVEQMHTDIISLWDQSLKPCVKLTPLCVTLNCSNVNVTTNIMKGEIKNCSFNMTTELRDKKQKVYSLFYKLDVVQINKSNSSSQYRLINCNTSAITQACPKVSFEPIPIHYCAPAGFAILKCKDKEFNGTGPCKNVSTVQCTHGIKPVVSTQLLLNGSLAEEEVMIRSENITNNAKNIIVQLTKPVKINCTRPNNNTRKSIRIGPGQAFYATGDIIGDIRQAHCNVSRTEWNETLQKVAKQLRKYFNNKTIIFTNSSGGRLRITTHSFNCGGEFFYCNTSGLFNSTWNGNGTKKKNSTESNDTITLPCRIKQIINMWQRVGQAMYAPPIQGVIRCESNITGLLLTRDGGDNNSKNETFRPGGGDMRDNWRSELYKYKVVKIEPLGVAPTKAKRRVVEREKRAVGIGAVFLGFLGAAGSTMGAASITLTVQARQLLSGIVQQQSNLLRAIEAQQHLLKLTVWGIKQLQARVLAVERYLKDQQLLGIWGCSGKLICTTNVPWNSSWSNKSQSEIWDNMTWLQWDKEISNYTDIIYNLIEESQNQQEKNEQDLLALDKWANLWNWFDISNWLWYIKIFIMIVGGLIGLRIVFAVLSV

SEQ ID NO: 3 - DNA, 2734 bp, Artificial Sequence
  Subtype B consensus Envelope DNA sequence construct
ggatccgccaccatggactggacctggattctgttcctggtggccgccgccaccagagtgcacagcagagtgaagggcatccggaagaactaccagcacctgtggagatggggcaccatgctgctgggcatgctgatgatctgttctgccgccgagaagctgtgggtgaccgtgtactacggcgtgcctgtgtggaaggaggccaccaccaccctgttctgcgccagcgacgccaaggcctacgataccgaagtgcacaatgtgtgggccacccacgcctgcgtgcctaccgatcccaaccctcaggaagtggtgctggagaacgtgaccgagaacttcaacatgtggaagaacaacatggtggagcagatgcacgaggacatcatcagcctgtgggaccagagcctgaagccttgcgtgaagctgacccctctgtgcgtgaccctgaactgcaccgacctgagcggcgagaagatggagaagggcgagatcaagaactgcagcttcaacatcaccacctccatccgggacaaagtgcagaaggagtacgccctgttctacaagctggacgtggtgcccatcgacaacgacaacaccagctaccggctgatcagctgcaacaccagcgtgatcacccaggcctgccccaaagtgagcttcgagcccatccccatccactactgcgcccctgccggcttcgccatcctgaagtgcaacgacaagaagttcaacggcaccggcccttgcaccaatgtgagcaccgtgcagtgcacccacggcatcagacccgtggtgtccacccagctgctgctgaacggcagcctggccgaggaagaagtggtgatccggagcgagaatttcaccaacaacgccaagaccatcatcgtgcagctgaacgagagcgtggagatcaactgcacccggcccaacaacaatacccggaagagcatccacatcggccctggccaggccttctacaccaccggcgagatcatcggcgatatcaggcaggcccactgcaatatcagccgggccaagtggaacaacaccctgaagcagatcgtgaagaagctgcgggagcagttcggcaacaagaccatcgtgttcaaccagagcagcggcggcagacctagaatcgtgatgcacagcttcaactgtggcggcgagttcttctactgcaacacaacccagctgttcaacagcacctggaacgtgaacgggacctggaacaacaacaccgagggcaacgacaccatcaccctgccctgccggatcaagcagatcatcaatatgtggcaggaggtgggcaaggccatgtacgcccctcccatcagaggccagatccggtgcagcagcaatatcaccggcctgctgctgaccagagatggcggcaacaataacaccaacgagaccgagatctttagacctggcggcggagacatgagggacaactggcggagcgagctgtacaagtacaaagtggtgaagatcgagcccctgggcgtggcccccaccaaggccaagagaagagtggtgcagcgggagaagagagctgtgggcatcggcgccatgtttctgggctttctgggagccgccggaagcaccatgggagccgccagcatgaccctgaccgtgcaggccagacagctgctgagcggcatcgtgcagcagcagaacaacctgctgagagccatcgaggcccagcagcacctgctgcagctgacagtgtggggcatcaagcagctgcaggcccgcgtgctggccgtggagagatacctgaaggaccagcagctgctgggaatctggggctgcagcggcaagctgatctgcaccaccaccgtgccctggaacgccagctggagcaacaagagcctggacgagatctgggacaacatgacctggatggagtgggagcgggagatcgacaactacaccagcctgatctacaccctgatcgaggagagccagaaccagcaggagaagaacgagcaggagctgctggagctggacaagtgggccagcctgtggaactggttcgacatcaccaactggctgtggtacatcaagatcttcatcatgattgtgggcggcctgatcggcctgagaatcgtgttcgccgtgctgagcatctacccctacgacgtgcccgattacgcctgagaattcgtaagtaagtgtcatatgggagagctcgactagactggacagccaatgacgggtaagagagtgacatttctcactaacctaagacaggagggccgtcaaagctactgcctaatccaatgacgggtaatagtgacaagaaatgtatcactccaacctaagacaggcgcagcctccgagggatgtgtcttttgttttttataattaaaaagggtgacatgtccggagccgtgctgcccggatgatgtcttggcctctgtttgctaccggtatcgatgttaacgtcgaccccgggctcgaggtaagtaagtgtcatatgggagagctcgactagactggacagccaatgacgggtaagagagtgacatttctcactaacctaagacaggagggccgtcaaagctactgcctaatccaatgacgggtaatagtgacaagaaatgtatcactccaacctaagacaggcgcagcctccgagggatgtgtcttttgttttttataattaaaaagggtgacatgtccggagccgtgctgcccggatgatgtcttggcctctgtttgctgcggccgc

SEQ ID NO: 4 - protein, 715 aa, Artificial Sequence
  Subtype B consensus Envelope protein sequence construct
MDWTWILFLVAAATRVHSRVKGIRKNYQHLWRWGTMLLGMLMICSAAEKLWVTVYYGVPVWKEATTTLFCASDAKAYDTEVHNVWATHACVPTDPNPQEVVLENVTENFNMWKNNMVEQMHEDIISLWDQSLKPCVKLTPLCVTLNCTDLSGEKMEKGEIKNCSFNITTSIRDKVQKEYALFYKLDVVPIDNDNTSYRLISCNTSVITQACPKVSFEPIPIHYCAPAGFAILKCNDKKFNGTGPCTNVSTVQCTHGIRPVVSTQLLLNGSLAEEEVVIRSENFTNNAKTIIVQLNESVEINCTRPNNNTRKSIHIGPGQAFYTTGEIIGDIRQAHCNISRAKWNNTLKQIVKKLREQFGNKTIVFNQSSGGRPRIVMHSFNCGGEFFYCNTTQLFNSTWNVNGTWNNNTEGNDTITLPCRIKQIINMWQEVGKAMYAPPIRGQIRCSSNITGLLLTRDGGNNNTNETEIFRPGGGDMRDNWRSELYKYKVVKIEPLGVAPTKAKRRVVQREKRAVGIGAMFLGFLGAAGSTMGAASMTLTVQARQLLSGIVQQQNNLLRAIEAQQHLLQLTVWGIKQLQARVLAVERYLKDQQLLGIWGCSGKLICTTTVPWNASWSNKSLDEIWDNMTWMEWEREIDNYTSLIYTLIEESQNQQEKNEQELLELDKWASLWNWFDITNWLWYIKIFIMIVGGLIGLRIVFAVLSIYPYDVPDYA

SEQ ID NO: 5 - DNA, 2140 bp, Artificial Sequence
  Subtype C consensus Envelope DNA sequence construct
ggatccgccaccatggattggacctggattctgttcctggtggccgccgccacaagagtgcacagcagagtgcggggcatcctgagaaattgccagcagtggtggatctggggcattctggggttctggatgctgatgatctgcaacgtgatgggcaacctgtgggtgaccgtgtactacggcgtgcctgtgtggaaggaggccaagaccaccctgttctgtgccagcgatgccaaggcctacgagaccgaggtgcacaatgtgtgggccacccacgcctgtgtgcccaccgatcccaaccctcaggagatggtgctggagaacgtgaccgagaacttcaacatgtggaagaacgacatggtggaccagatgcacgaggacatcatcagcctgtgggaccagagcctgaagccttgcgtgaagctgacccctctgtgcgtgaccctgaactgccggaacaacgtgaacaacaacaacaccatgaaggaggagatcaagaactgcagcttcaacatcaccaccgagctgcgggacaagaagcagaaggtgtacgccctgttctaccggctggacatcgtgcccctgaacgagaagaacaacagcaacgactaccggctgatcaactgcaacaccagcgccatcacccaggcctgtcccaaggtgtccttcgaccccatccccatccactattgtgcccctgccggctacgccatcctgaagtgcaacaacaagaccttcaacggcaccggcccctgcaataatgtgagcaccgtgcagtgtacccacggcatcaagcctgtggtgtccacccagctgctgctgaatggcagcctggccgaggaggagattatcatccggagcgagaacctgaccaacaacgccaagaccatcattgtgcacctgaatgagagcgtggagatcgtgtgtacccggcccaacaacaatacccggaagagcatcagaatcggccctggccagaccttttacgccaccggcgacatcatcggcgatatcaggcaggcccactgcaatatcagcgaggagaagtggaacaagaccctgcagcgggtgtccgagaagctgaaggagcacttccccaataagaccatcaagttcgcccctagcagcggcggcagactggagatcaccacccacagcttcaactgcaggggcgagttcttctactgcaataccagcaagctgttcaacagcacctacatgcccaacagcaccaacaataccaacaccaccatcaccctgccctgccggatcaagcagatcatcaatatgtggcaggaagtgggcagagccatgtacgcccctcccatcgagggcaacatcacctgcaagtccaacatcaccggcctgctgctgacaagagatggcggcaagaacgacaccaatgacaccgagaccttcagacctggcggcggagacatgagggacaactggcggagcgagctgtacaagtacaaggtggtggagatcaagcctctgggcgtggcccctaccaaggccaagaggagagtggtggagagggagaagagagccgtgggcatcggcgccgtgtttctgggctttctgggagccgccggatctacaatgggagccgccagcatcacactgaccgtgcaggccagacagctgctgagcggcatcgtgcagcagcagagcaatctgctgagagccatcgaggcccagcagcacatgctgcagctgacagtgtggggcatcaagcagctgcagaccagagtgctggccatcgagcgctacctgaaggatcagcagctgctgggcatctggggctgtagcggcaagctgatctgtaccaccgccgtgccttggaatagcagctggagcaacaagagccaggaggacatctgggacaacatgacctggatgcagtgggaccgggagatcagcaactacaccgacaccatctacaggctgctggaggacagccagaaccagcaggagaagaacgagaaggacctgctggccctggacagctggaagaacctgtggaactggttcgacatcaccaactggctgtggtacatcaagatcttcatcatgattgtgggcggcctgatcggcctgagaatcatcttcgccgtgctgagcatctgatagcggccgc

SEQ ID NO: 6 - protein, 705 aa, Artificial Sequence
  Subtype C consensus Envelope protein sequence construct
MDWTWILFLVAAATRVHSRVRGILRNCQQWWIWGILGFWMLMICNVMGNLWVTVYYGVPVWKEAKTTLFCASDAKAYETEVHNVWATHACVPTDPNPQEMVLENVTENFNMWKNDMVDQMHEDIISLWDQSLKPCVKLTPLCVTLNCRNNVNNNNTMKEEIKNCSFNITTELRDKKQKVYALFYRLDIVPLNEKNNSNDYRLINCNTSAITQACPKVSFDPIPIHYCAPAGYAILKCNNKTFNGTGPCNNVSTVQCTHGIKPVVSTQLLLNGSLAEEEIIIRSENLTNNAKTIIVHLNESVEIVCTRPNNNTRKSIRIGPGQTFYATGDIIGDIRQAHCNISEEKWNKTLQRVSEKLKEHFPNKTIKFAPSSGGRLEITTHSFNCRGEFFYCNTSKLFNSTYMPNSTNNTNTTITLPCRIKQIINMWQEVGRAMYAPPIEGNITCKSNITGLLLTRDGGKNDTNDTETFRPGGGDMRDNWRSELYKYKVVEIKPLGVAPTKAKRRVVEREKRAVGIGAVFLGFLGAAGSTMGAASITLTVQARQLLSGIVQQQSNLLRAIEAQQHMLQLTVWGIKQLQTRVLAIERYLKDQQLLGIWGCSGKLICTTAVPWNSSWSNKSQEDIWDNMTWMQWDREISNYTDTIYRLLEDSQNQQEKNEKDLLALDSWKNLWNWFDITNWLWYIKIFIMIVGGLIGLRIIFAVLSI

SEQ ID NO: 7 - DNA, 2089 bp, Artificial Sequence
  Subtype D consensus Envelope DNA sequence construct
gggcatcaagcggaattaccagcacctgtggaagtggggcaccatgctgctgggcatgctgatgacctgcagcgtggccgagaacctgtgggtgaccgtgtactacggcgtgcctgtgtggaaggaagccaccaccaccctgttctgcgccagcgatgccaagagctacaagaccgaggcccacaatatctgggccacccacgcctgcgtgcctaccgatcccaaccctcaggagatcgagctggagaacgtgaccgagaacttcaacatgtggaagaacaacatggtggagcagatgcacgaggacatcatcagcctgtgggaccagagcctgaagccttgcgtgaagctgacccctctgtgcgtgaccctgaactgcaccgacggcatgaggaacgacaccaacgataccaacgtgaccatggaggagggcgagatgaagaactgcagcttcaacatcaccaccgaagtgcgggacaagaagaagcaggtgcacgccctgttctacaagctggacgtggtgcccatcgacgacaacaacaccaacaacagcaactaccggctgatcaactgcaacaccagcgccatcacccaggcctgccccaaagtgaccttcgagcccatccccatccactactgcgcccctgccggcttcgccatcctgaagtgcaaggataagaagttcaacggcaccggcccctgcaagaatgtgagcaccgtgcagtgcacccacggcatcagacccgtggtgtccacccagctgctgctgaacggcagcctggccgaggaggagatcatcatccggagcgagaacctgaccaacaacgccaagatcatcattgtgcagctgaacgagagcgtgaccatcaattgcacccggccctacaacaatacccggaagcgcatccccatcggcctgggccaggccttctacaccaccagaggcatcatcggcgacatcagacaggcccactgcaatatcagcggagccgagtggaataagaccctgcagcaggtggccaagaagctgggcgacctgctgaacaagaccaccatcatcttcaagcctagcagcggcggcagacctagaatcaccacccacagcttcaattgtggcggcgagttcttctactgcaataccagccggctgttcaacagcacctggagcaagaacagcaccagcaactccaccaaggagaacaacaccatcaccctgccctgccggatcaagcagatcatcaatatgtggcagggagtgggcaaggccatgtacgcccctcccatcgagggcctgatcaagtgcagcagcaacatcaccggcctgctgctgaccagagatggcggagccaacaactcccacaacgagaccttcagacctggcggcggagacatgagggacaactggcggagcgagctgtacaagtacaaagtggtgaagatcgagcccctgggcgtggcccccaccagagccaagagaagagtggtggagcgggagaagagagccatcggactgggcgccatgttcctgggcttcctgggagccgccggaagcaccatgggagccgccagcctgaccctgaccgtgcaggccagacagctgctgagcggcatcgtgcagcagcagaacaacctgctgagagccattgaggcccagcagcacctgctgcagctgacagtgtggggcattaagcagctgcaggccaggattctggccgtggagcgctacctgaaggatcagcagctgctgggaatctggggctgcagcggcaagcacatctgcaccaccaccgtgccttggaatagcagctggagcaacaagagcctggacgagatctggaacaacatgacctggatggagtgggagagggagatcgacaactacaccggcctgatctacagcctgatcgaggagagccagacccagcaggagaagaacgagcaggagctgctggagctggacaagtgggccagcctgtggaactggttcagcatcacccagtggctgtggtacatcaagatcttcatcatgattgtgggcggcctgatcggcctgagaatcgtgttcgccgtgctgagcctgtgactcgag

SEQ ID NO: 8 - protein, 714 aa, Artificial Sequence
  Subtype D consensus Envelope protein sequence construct
MDWTWILFLVAAATRVHSRVRGIKRNYQHLWKWGTMLLGMLMTCSVAENLWVTVYYGVPVWKEATTTLFCASDAKSYKTEAHNIWATHACVPTDPNPQEIELENVTENFNMWKNNMVEQMHEDIISLWDQSLKPCVKLTPLCVTLNCTDGMRNDTNDTNVTMEEGEMKNCSFNITTEVRDKKKQVHALFYKLDVVPIDDNNTNNSNYRLINCNTSAITQACPKVTFEPIPIHYCAPAGFAILKCKDKKFNGTGPCKNVSTVQCTHGIRPVVSTQLLLNGSLAEEEIIIRSENLTNNAKIIIVQLNESVTINCTRPYNNTRKRIPIGLGQAFYTTRGIIGDIRQAHCNISGAEWNKTLQQVAKKLGDLLNKTTIIFKPSSGGRPRITTHSFNCGGEFFYCNTSRLFNSTWSKNSTSNSTKENNTITLPCRIKQIINMWQGVGKAMYAPPIEGLIKCSSNITGLLLTRDGGANNSHNETFRPGGGDMRDNWRSELYKYKVVKIEPLGVAPTRAKRRVVEREKRAIGLGAMFLGFLGAAGSTMGAASLTLTVQARQLLSGIVQQQNNLLRAIEAQQHLLQLTVWGIKQLQARILAVERYLKDQQLLGIWGCSGKHICTTTVPWNSSWSNKSLDEIWNNMTWMEWEREIDNYTGLIYSLIEESQTQQEKNEQELLELDKWASLWNWFSITQWLWYIKIFIMIVGGLIGLRIVFAVLSL

SEQ ID NO: 9 - DNA, 1049 bp, Artificial Sequence
  Subtype B consensus Nef-Rev DNA sequence construct
ggatccgccaccatggactggacctggattctgttcctggtggccgctgccaccagagtgcacagcagcaagagaagcgtggtgggttggcctacagtgcgggagaggatgagaagagccgagcctgccgccgatggagtgggcgccgtgtctagagatctggagaagcacggcgccatcaccagcagcaataccgccgccaacaatgccgactgcgcctggctggaggcccaggaggaggaggaagtgggcttccctgtgagagcccaggtggccctgagagccatgacctacaaggccgccgtggatctgagccacttcctgaaggagaagggcggcctggagggcctgatctacagccagaagcggcaggacatcctggatctgtgggtgtaccacacccagggctacttccccgactggcagaattacacccctggccctggcatcagataccctctgaccttcggctggtgcttcaagctggtgcctgtggagcctgagaaagtggaggaggccaacgagggcgagaacaattctgccgcccaccctatgagcctgcacggcatggacgatcccgagagggaagtgctggtgtggaagttcgacagcaggctggccttccaccacatggccagagagctgcaccccgagtactacaaggactgccggggcaggaagagaagaagcgccggcagaagcggcgacagcgacgaggagctgctgaaaacagtgcggctgatcaagttcctgtaccagagcaaccctcctcccagccccgagggcaccagacaggcccggagaaaccggaggaggcggtggagagagaggcagcggcagatcagaagcatcagcgagtggattctgagcacctacctgggcagacccgccgagcccgtgcccctgcagctgccccccctggagagactgaccctggactgcaacgaggactgcggcaccagcggcacccagggagtgggcagcccccagatcctggtggagagccctgccgtgctggagagcggcaccaaggagtgatgagcggccgc

SEQ ID NO: 10 - protein, 341 aa, Artificial Sequence
  Subtype B consensus Nef-Rev protein sequence construct
MDWTWILFLVAAATRVHSSKRSVVGWPTVRERMRRAEPAADGVGAVSRDLEKHGAITSSNTAANNADCAWLEAQEEEEVGFPVRAQVALRAMTYKAAVDLSHFLKEKGGLEGLIYSQKRQDILDLWVYHTQGYFPDWQNYTPGPGIRYPLTFGWCFKLVPVEPEKVEEANEGENNSAAHPMSLHGMDDPEREVLVWKFDSRLAFHHMARELHPEYYKDCRGRKRRSAGRSGDSDEELLKTVRLIKFLYQSNPPPSPEGTRQARRNRRRRWRERQRQIRSISEWILSTYLGRPAEPVPLQLPPLERLTLDCNEDCGTSGTQGVGSPQILVESPAVLESGTKE

SEQ ID NO: 11 - DNA, 1863 bp, Artificial Sequence
  Gag consensus DNA sequence of subtype A, B, C and D construct
ggatccgccaccatggactggacctggattctgtttctggtcgccgccgccacaagagtgcacagcggcgccagagccagcgtgctgtccggcggcaagctggacgcctgggagaagatcagactgaggcctggcggcaagaagaagtaccggctgaagcaccttgtgtgggccagcagagagctggagagattcgccctgaatcctggcctgctggagaccagcgagggctgtaagcagatcatcggccagctgcagcccgccctgcagaccggcagcgaggagctgagaagcctgtacaacaccgtggccaccctgtactgcgtgcacgagaagatcgaggtgaaggacaccaaggaggccctggacaagatcgaggaggagcagaacaagagcaagcagaaggcccagcaggccgccgccgacaccggcaacagcagccaggtgtcccagaactaccccatcgtgcagaatctgcagggccagatggtgcaccaggccatcagccccagaaccctgaatgcctgggtgaaggtgatcgaggagaaggccttcagccctgaggtgatccctatgttcagcgccctgagcgagggcgccacacctcaggacctgaacaccatgctgaacacagtggggggccaccaggccgccatgcagatgctgaaggataccatcaacgaggaggccgccgagtgggacagactgcaccccgtgcacgccggacctatcgcccctggccagatgagagagcccagaggcagcgacatcgccggcaccacctccaccctgcaagagcagatcggctggatgaccagcaacccccccatccctgtgggcgacatctacaagcggtggatcatcctgggcctgaacaagattgtgaggatgtacagccccgtgtccatcctggatatcaggcagggccccaaggagcccttcagagactacgtggaccggttcttcaagaccctgagagccgagcaggccagccaggacgtgaagaactggatgaccgagaccctgctggtgcagaacgccaaccccgactgtaagaccatcctgagagccctgggccctggcgccaccctggaggagatgatgaccgcctgccagggagtgggcggacccggccacaaggccagagtgctggccgaggccatgagccaggccaccaacagcaacatcatgatgcagcggggcaacttcagaggccccaggaggatcgtgaagtgcttcaactgtggcaaggagggccacatcgccagaaactgtagggcccccaggaagaagggctgctggaagtgtggcaaagaggggcaccagatgaaggactgtaccgagcggcaggccaatttcctggggaagatctggcccagccacaagggcagacccggcaatttcctgcagagcagacctgagcccaccgcccctcccgccgagagcttcggcttcggcgaggagatcacccccagccccaagcaggagcccaaggacagagagctgtaccctctggccagcctgaagagcctgttcggcaacgatcccctgagccagtacccctacgacgtgcccgattacgcctgagaattcgtaagtaagtgtcatatgggagagctcgactagactggacagccaatgacgggtaagagagtgacatttctcactaacctaagacaggagggccgtcaaagctactgcctaatccaatgacgggtaatagtgacaagaaatgtatcactccaacctaagacaggcgcagcctccgagggatgtgtcttttgttttttataattaaaaagggtgacatgtccggagccgtgctgcccggatgatgtcttggcctctgtttgctgcggccgc

SEQ ID NO: 12 - protein, 524 aa, Artificial Sequence
  Gag consensus protein sequence of subtype A, B, C and D construct
MDWTWILFLVAAATRVHSGARASVLSGGKLDAWEKIRLRPGGKKKYRLKHLVWASRELERFALNPGLLETSEGCKQIIGQLQPALQTGSEELRSLYNTVATLYCVHEKIEVKDTKEALDKIEEEQNKSKQKAQQAAADTGNSSQVSQNYPIVQNLQGQMVHQAISPRTLNAWVKVIEEKAFSPEVIPMFSALSEGATPQDLNTMLNTVGGHQAAMQMLKDTINEEAAEWDRLHPVHAGPIAPGQMREPRGSDIAGTTSTLQEQIGWMTSNPPIPVGDIYKRWIILGLNKIVRMYSPVSILDIRQGPKEPFRDYVDRFFKTLRAEQASQDVKNWMTETLLVQNANPDCKTILRALGPGATLEEMMTACQGVGGPGHKARVLAEAMSQATNSNIMMQRGNFRGPRRIVKCFNCGKEGHIARNCRAPRKKGCWKCGKEGHQMKDCTERQANFLGKIWPSHKGRPGNFLQSRPEPTAPPAESFGFGEEITPSPKQEPKDRELYPLASLKSLFGNDPLSQYPYDVPDYA

SEQ ID NO: 13 - DNA, 43 bp, Artificial Sequence
  IgE Primer Sequence 1
gtcgctccgctagcttgtgggtcacagtctattatggggtacc

SEQ ID NO: 14 - DNA, 35 bp, Artificial Sequence
  IgE Primer Sequence 2
ggtcggatccttactccaccactctcctttttgcc

SEQ ID NO: 15 - protein, 17 aa, Artificial Sequence
  IgE leader sequence
MDWTWILFLVAAATRVH

SEQ ID NO: 16 - protein, 692 aa, Artificial Sequence
  Subtype A consensus Envelope protein sequence
SRVMGIQRNCQHLWRWGTMILGMIIICSAAENLWVTVYYGVPVWKDAETTLFCASDAKAYDTEVHNVWATHACVPTDPNPQEINLENVTEEFNMWKNNMVEQMHTDIISLWDQSLKPCVKLTPLCVTLNCSNVNVTTNIMKGEIKNCSFNMTTELRDKKQKVYSLFYKLDVVQINKSNSSSQYRLINCNTSAITQACPKVSFEPIPIHYCAPAGFAILKCKDKEFNGTGPCKNVSTVQCTHGIKPVVSTQLLLNGSLAEEEVMIRSENITNNAKNIIVQLTKPVKINCTRPNNNTRKSIRIGPGQAFYATGDIIGDIRQAHCNVSRTEWNETLQKVAKQLRKYFNNKTIIFTNSSGGRLRITTHSFNCGGEFFYCNTSGLFNSTWNGNGTKKKNSTESNDTITLPCRIKQIINMWQRVGQAMYAPPIQGVIRCESNITGLLLTRDGGDNNSKNETFRPGGGDMRDNWRSELYKYKVVKIEPLGVAPTKAKRRVVEREKRAVGIGAVFLGFLGAAGSTMGAASITLTVQARQLLSGIVQQQSNLLRAIEAQQHLLKLTVWGIKQLQARVLAVERYLKDQQLLGIWGCSGKLICTTNVPWNSSWSNKSQSEIWDNMTWLQWDKEISNYTDIIYNLIEESQNQQEKNEQDLLALDKWANLWNWFDISNWLWYIKIFIMIVGGLIGLRIVFAVLSV

SEQ ID NO: 17 - protein, 697 aa, Artificial Sequence
  Subtype B consensus Envelope protein sequence
RVKGIRKNYQHLWRWGTMLLGMLMICSAAEKLWVTVYYGVPVWKEATTTLFCASDAKAYDTEVHNVWATHACVPTDPNPQEVVLENVTENFNMWKNNMVEQMHEDIISLWDQSLKPCVKLTPLCVTLNCTDLSGEKMEKGEIKNCSFNITTSIRDKVQKEYALFYKLDVVPIDNDNTSYRLISCNTSVITQACPKVSFEPIPIHYCAPAGFAILKCNDKKFNGTGPCTNVSTVQCTHGIRPVVSTQLLLNGSLAEEEVVIRSENFTNNAKTIIVQLNESVEINCTRPNNNTRKSIHIGPGQAFYTTGEIIGDIRQAHCNISRAKWNNTLKQIVKKLREQFGNKTIVFNQSSGGRPRIVMHSFNCGGEFFYCNTTQLFNSTWNVNGTWNNNTEGNDTITLPCRIKQIINMWQEVGKAMYAPPIRGQIRCSSNITGLLLTRDGGNNNTNETEIFRPGGGDMRDNWRSELYKYKVVKIEPLGVAPTKAKRRVVQREKRAVGIGAMFLGFLGAAGSTMGAASMTLTVQARQLLSGIVQQQNNLLRAIEAQQHLLQLTVWGIKQLQARVLAVERYLKDQQLLGIWGCSGKLICTTTVPWNASWSNKSLDEIWDNMTWMEWEREIDNYTSLIYTLIEESQNQQEKNEQELLELDKWASLWNWFDITNWLWYIKIFIMIVGGLIGLRIVFAVLSIYPYDVPDYA

SEQ ID NO: 18 - protein, 687 aa, Artificial Sequence
  Subtype C consensus Envelope protein sequence
RVRGILRNCQQWWIWGILGFWMLMICNVMGNLWVTVYYGVPVWKEAKTTLFCASDAKAYETEVHNVWATHACVPTDPNPQEMVLENVTENFNMWKNDMVDQMHEDIISLWDQSLKPCVKLTPLCVTLNCRNNVNNNNTMKEEIKNCSFNITTELRDKKQKVYALFYRLDIVPLNEKNNSNDYRLINCNTSAITQACPKVSFDPIPIHYCAPAGYAILKCNNKTFNGTGPCNNVSTVQCTHGIKPVVSTQLLLNGSLAEEEIIIRSENLTNNAKTIIVHLNESVEIVCTRPNNNTRKSIRIGPGQTFYATGDIIGDIRQAHCNISEEKWNKTLQRVSEKLKEHFPNKTIKFAPSSGGRLEITTHSFNCRGEFFYCNTSKLFNSTYMPNSTNNTNTTITLPCRIKQIINMWQEVGRAMYAPPIEGNITCKSNITGLLLTRDGGKNDTNDTETFRPGGGDMRDNWRSELYKYKVVEIKPLGVAPTKAKRRVVEREKRAVGIGAVFLGFLGAAGSTMGAASITLTVQARQLLSGIVQQQSNLLRAIEAQQHMLQLTVWGIKQLQTRVLAIERYLKDQQLLGIWGCSGKLICTTAVPWNSSWSNKSQEDIWDNMTWMQWDREISNYTDTIYRLLEDSQNQQEKNEKDLLALDSWKNLWNWFDITNWLWYIKIFIMIVGGLIGLRIIFAVLSI

SEQ ID NO: 19 - protein, 696 aa, Artificial Sequence
  Subtype D consensus Envelope protein sequence
RVRGIKRNYQHLWKWGTMLLGMLMTCSVAENLWVTVYYGVPVWKEATTTLFCASDAKSYKTEAHNIWATHACVPTDPNPQEIELENVTENFNMWKNNMVEQMHEDIISLWDQSLKPCVKLTPLCVTLNCTDGMRNDTNDTNVTMEEGEMKNCSFNITTEVRDKKKQVHALFYKLDVVPIDDNNTNNSNYRLINCNTSAITQACPKVTFEPIPIHYCAPAGFAILKCKDKKFNGTGPCKNVSTVQCTHGIRPVVSTQLLLNGSLAEEEIIIRSENLTNNAKIIIVQLNESVTINCTRPYNNTRKRIPIGLGQAFYTTRGIIGDIRQAHCNISGAEWNKTLQQVAKKLGDLLNKTTIIFKPSSGGRPRITTHSFNCGGEFFYCNTSRLFNSTWSKNSTSNSTKENNTITLPCRIKQIINMWQGVGKAMYAPPIEGLIKCSSNITGLLLTRDGGANNSHNETFRPGGGDMRDNWRSELYKYKVVKIEPLGVAPTRAKRRVVEREKRAIGLGAMFLGFLGAAGSTMGAASLTLTVQARQLLSGIVQQQNNLLRAIEAQQHLLQLTVWGIKQLQARILAVERYLKDQQLLGIWGCSGKHICTTTVPWNSSWSNKSLDEIWNNMTWMEWEREIDNYTGLIYSLIEESQTQQEKNEQELLELDKWASLWNWFSITQWLWYIKIFIMIVGGLIGLRIVFAVLSL

SEQ ID NO: 20 - protein, 323 aa, Artificial Sequence
  Subtype B consensus Nef-Rev protein sequence
SKRSVVGWPTVRERMRRAEPAADGVGAVSRDLEKHGAITSSNTAANNADCAWLEAQEEEEVGFPVRAQVALRAMTYKAAVDLSHFLKEKGGLEGLIYSQKRQDILDLWVYHTQGYFPDWQNYTPGPGIRYPLTFGWCFKLVPVEPEKVEEANEGENNSAAHPMSLHGMDDPEREVLVWKFDSRLAFHHMARELHPEYYKDCRGRKRRSAGRSGDSDEELLKTVRLIKFLYQSNPPPSPEGTRQARRNRRRRWRERQRQIRSISEWILSTYLGRPAEPVPLQLPPLERLTLDCNEDCGTSGTQGVGSPQILVESPAVLESGTKE

SEQ ID NO: 21 - protein, 506 aa, Artificial Sequence
  Gag consensus protein sequence of subtype A, B, C and D
GARASVLSGGKLDAWEKIRLRPGGKKKYRLKHLVWASRELERFALNPGLLETSEGCKQIIGQLQPALQTGSEELRSLYNTVATLYCVHEKIEVKDTKEALDKIEEEQNKSKQKAQQAAADTGNSSQVSQNYPIVQNLQGQMVHQAISPRTLNAWVKVIEEKAFSPEVIPMFSALSEGATPQDLNTMLNTVGGHQAAMQMLKDTINEEAAEWDRLHPVHAGPIAPGQMREPRGSDIAGTTSTLQEQIGWMTSNPPIPVGDIYKRWIILGLNKIVRMYSPVSILDIRQGPKEPFRDYVDRFFKTLRAEQASQDVKNWMTETLLVQNANPDCKTILRALGPGATLEEMMTACQGVGGPGHKARVLAEAMSQATNSNIMMQRGNFRGPRRIVKCFNCGKEGHIARNCRAPRKKGCWKCGKEGHQMKDCTERQANFLGKIWPSHKGRPGNFLQSRPEPTAPPAESFGFGEEITPSPKQEPKDRELYPLASLKSLFGNDPLSQYPYDVPDYA

SEQ ID NO: 22 - DNA, 818 bp, Artificial Sequence
  HPV genotype 16 E6-E7 DNA sequence
gaattcgccaccatggactggacctggatcctgttcctggtggccgccgccacacgggtgcacagcttccaggacccccaggagagcggcagaaagctgcctcagctgtgtaccgagctgcagaccaccatccacgacatcatcctggagtgtgtgtactgtaagcagcagctgctgaggagagaggtgtacgaccgggacctgtgtatcgtgtacagggacggcaatccctacgccgtgtgtgacaagtgcctgaagttctacagcaagatcagcgagtaccggcactactgctacagcctgtacggcaccaccctggagcagcagtacaacaagcccctgtgtgacctgctgatccggtgtatcaactgccagaagcccctgcagagacacctggacaagaagcagcggttccacaacatcaggggcagatggaccggcagatgtatgagctgctgccggagcagcagaaccagaagggagacccagctgagaggccggaagagaagaagccacggcgatacccccaccctgcacgagtacatgctggacctgcagcctgagaccaccgatctgtacggctacggccagctgaatgacagcagcgaggaggaggatgagatcgacggccctgccggccaggccgagcccgacagagcccactacaacatcgtgaccttttgctgtaagtgtgacagcaccctgagactgtgcgtgcagagcacccacgtggacatcagaaccctggaggatctgctgatgggcaccctgggcatcgtgtgtcccatctgctcccagaaaccctgatgagcggccgc

SEQ ID NO: 23 - protein, 264 aa, Artificial sequence
  HPV genotype 16 E6-E7 protein sequence
MDWTWILFLVAAATRVHSFQDPQESGRKLPQLCTELQTTIHDIILECVYCKQQLLRREVYDRDLCIVYRDGNPYAVCDKCLKFYSKISEYRHYCYSLYGTTLEQQYNKPLCDLLIRCINCQKPLQRHLDKKQRFHNIRGRWTGRCMSCCRSSRTRRETQLRGRKRRSHGDTPTLHEYMLDLQPETTDLYGYGQLNDSSEEEDEIDGPAGQAEPDRAHYNIVTFCCKCDSTLRLCVQSTHVDIRTLEDLLMGTLGIVCPICSQKP

SEQ ID NO: 24 - protein, 15 aa, Artificial Sequence
  HPV E6 immunodominant epitope
LCIVYRDGNPYAVCD

SEQ ID NO: 25 - protein, 15 aa, Artificial Sequence
  HPV E7 immunodominant epitope
AEPDRAHYNIVTFCC

SEQ ID NO: 26 - protein, 142 aa, Artificial Sequence
  HPV E6 consensus sequence
FQDPQESGRKLPQLCTELQTTIHDIILECVYCKQQLLRREVYDRDLCIVYRDGNPYAVCDKCLKFYSKISEYRHYCYSLYGTTLEQQYNKPLCDLLIRCINCQKPLQRHLDKKQRFHNIRGRWTGRCMSCCRSSRTRRETQL

SEQ ID NO: 27 - protein, 97 aa, Artificial Sequence
  HPV E7 consensus sequence
HGDTPTLHEYMLDLQPETTDLYGYGQLNDSSEEEDEIDGPAGQAEPDRAHYNIVTFCCKCDSTLRLCVQSTHVDIRTLEDLLMGTLGIVCPICSQKP

SEQ ID NO: 28 - protein, 18 aa, Artificial Sequence
  IgE Leader Sequence
MDWTWILFLVAAATRVHS

SEQ ID NO: 29 - protein, 7 aa, Artificial Sequence
  Proteolytic Cleavage Sequence
RGRKRRS

SEQ ID NO: 30 - DNA, 1766 bp, Artificial Sequence
  HCV genotype 1a and 1b consensus E1-E2 DNA sequence
gaattcgccaccatggactggacctggatcctgttcctggtggccgctgcaacacgggtgcacagctaccaagtgaggaatagcagcggcctgtaccacgtgaccaacgactgctccaacagcagcatcgtgtacgaggccgccgacatgatcatgcacacccccggctgtgtgccctgtgtgagagagggcaacagctccagatgctgggtggccctgacccctaccgtggccgccagagatggcagcctgcccaccaccaccctgaggagacacgtggacctgcttgtgggcagcgccaccctgtgtagcgccatgtatgtgggcgatctgtgtggcagcgtgtttcttgtgggccagctgttcaccttcagccccagaaggcactggaccgtgcaggactgtaactgctccatctaccccggccacatcaccggccacagaatggcctgggacatgatgatgaactggagccctaccaccgccctggtggtgtcccagctgctgagaatccctcaggccatcgtggacatggtggccggagcccactggggcgtgctggccggcatcgcctacttcagcatggtgggcaactgggccaaggtgctcgtggtgctgctgctgttcgccggcgtggacggcagaggcaggaagagaaggagcgagacccacgtgaccggcggcaccgccggcagaaccacagccggccttgtgggcctgttcacccctggcgccaagcagaacatccagctgatcaacaccaacggcagctggcacatcaacagcaccgccctgaactgtaacgacagcctgaacaccggctggctggccggcctgttctaccagcacaagttcaacagcagcggctgccccgagagaatggccagctgtagacccctggatgagttcgcccagggctggggccccatcacctacgccaatggcagcggccctgaccagagaccctactgctggcactacgcccccagaccctgtggcatcgtgcccgccaagagcgtgtgtggccccgtgtactgcttcacccctagccccgtggttgtgggcaccaccgacagaagcggagcccccacctacagctggggcgagaacgagaccgacgtgctggtgctgaacaacaccagaccccccctgggcaattggttcggctgtacctggatgaacagcaccggcttcaccaaagtgtgtggcgcccctccctgtgtgatcggcggagtgggcaacaacaccctgacctgccccaccgactgcttcagaaagcaccccgaggccacctactccagatgtggcagcggaccttggctgacccccagatgtatggtggactacccctacaggctgtggcactacccctgtaccgtgaacttcaccatcttcaaagtgaggatgtatgtggggggcgtggagcacagactggaggccgcctgtaattggaccaggggcgagagatgtgacctggaggaccgggatagaagcgagctgtcccctctgctgctgtccaccaccgagtggcaggtgctgccttgtagcttcaccaccctgcccgccctgagcaccggcctgatccacctgcaccagaacatcgtggacgtgcagtacctgtacggagtgggctctagcatcgtgtcctgggccatcaagtgggagtacgtggtgctgctgttcctgctgctggccgacgccagagtgtgtagctgcctgtggatgatgctgctgatcagccaggccgaggcctgatgagcggccgc

SEQ ID NO: 31 - protein, 580 aa, Artificial Sequence
  HCV genotype 1a and 1b consensus E1-E2 protein sequence
MDWTWILFLVAAATRVHSYQVRNSSGLYHVTNDCSNSSIVYEAADMIMHTPGCVPCVREGNSSRCWVALTPTVAARDGSLPTTTLRRHVDLLVGSATLCSAMYVGDLCGSVFLVGQLFTFSPRRHWTVQDCNCSIYPGHITGHRMAWDMMMNWSPTTALVVSQLLRIPQAIVDMVAGAHWGVLAGIAYFSMVGNWAKVLVVLLLFAGVDGRGRKRRSETHVTGGTAGRTTAGLVGLFTPGAKQNIQLINTNGSWHINSTALNCNDSLNTGWLAGLFYQHKFNSSGCPERMASCRPLDEFAQGWGPITYANGSGPDQRPYCWHYAPRPCGIVPAKSVCGPVYCFTPSPVVVGTTDRSGAPTYSWGENETDVLVLNNTRPPLGNWFGCTWMNSTGFTKVCGAPPCVIGGVGNNTLTCPTDCFRKHPEATYSRCGSGPWLTPRCMVDYPYRLWHYPCTVNFTIFKVRMYVGGVEHRLEAACNWTRGERCDLEDRDRSELSPLLLSTTEWQVLPCSFTTLPALSTGLIHLHQNIVDVQYLYGVGSSIVSWAIKWEYVVLLFLLLADARVCSCLWMMLLISQAEA

SEQ ID NO: 32 - protein, 192 aa, Artificial Sequence
  HCV E1 consensus sequence
YQVRNSSGLYHVTNDCSNSSIVYEAADMIMHTPGCVPCVREGNSSRCWVALTPTVAARDGSLPTTTLRRHVDLLVGSATLCSAMYVGDLCGSVFLVGQLFTFSPRRHWTVQDCNCSIYPGHITGHRMAWDMMMNWSPTTALVVSQLLRIPQAIVDMVAGAHWGVLAGIAYFSMVGNWAKVLVVLLLFAGVDG

SEQ ID NO: 33 - protein, 363 aa, Artificial Sequence
  HCV E2 consensus sequence
ETHVTGGTAGRTTAGLVGLFTPGAKQNIQLINTNGSWHINSTALNCNDSLNTGWLAGLFYQHKFNSSGCPERMASCRPLDEFAQGWGPITYANGSGPDQRPYCWHYAPRPCGIVPAKSVCGPVYCFTPSPVVVGTTDRSGAPTYSWGENETDVLVLNNTRPPLGNWFGCTWMNSTGFTKVCGAPPCVIGGVGNNTLTCPTDCFRKHPEATYSRCGSGPWLTPRCMVDYPYRLWHYPCTVNFTIFKVRMYVGGVEHRLEAACNWTRGERCDLEDRDRSELSPLLLSTTEWQVLPCSFTTLPALSTGLIHLHQNIVDVQYLYGVGSSIVSWAIKWEYVVLLFLLLADARVCSCLWMMLLISQAEA

SEQ ID NO: 34 - DNA, 3512 bp, Homo sapiens
ggtaccgaattcgccaccatggactggacctggatcctgttcctggtggccgctgccacaagagtgcacagccccagggcccccaggtgcagagccgtgcggagcctgctgcggagccactaccgggaggtgctgcccctggccaccttcgtgcggaggctgggccctcaggggtggcggctggtgcagagaggcgaccctgccgccttcagagccctggtggcccagtgcctggtgtgcgtgccctgggacgccagacctccccctgccgcccctagcttccggcaggtgtcctgcctgaaagaactggtggcccgggtgctgcagcggctgtgcgagaggggcgccaagaacgtgctggccttcggcttcgccctgctggacggcgccagaggcggccctcccgaggccttcaccacctccgtgagaagctacctgcccaacaccgtgaccgacgccctgagaggcagcggcgcttggggcctgctgctgcgcagagtgggcgacgacgtgctggtgcacctgctggccagatgcgccctgttcgtgctggtcgcccccagctgcgcctaccaggtgtgcggcccacccctgtaccagctgggagccgccacccaggccagaccccctcctcacgcctccggccccaggcggagactgggctgcgagcgggcctggaaccacagcgtgcgggaggccggcgtgcccctgggcctgccagcccctggcgccagaagaaggggcggcagcgccagcagaagcctgcccctgcccaagcggcccagacgcggagccgcccctgagcccgagagaacccccgtgggccagggctcttgggcccaccctggccggaccagaggccccagcgaccggggcttctgcgtggtgtcccccgccagacccgccgaggaagccacctccctggaaggcgccctgagcggcaccaggcacagccaccccagcgtgggccgccagcaccacgccggaccccccagcacctccaggccccccaggccctgggacaccccttgcccccctgtgtacgccgagaccaagcacttcctgtacagcagcggcgacaaagagcagctgcggcccagcttcctgctgtccagcctgaggccctccctgaccggcgctaggcgcctggtggagaccatctttctgggcagccggccctggatgcccggcacccccaggcggctgcccaggctgccccagcggtactggcagatgaggcctctgttcctggaactgctgggcaaccacgcccagtgcccctacggcgtgctgctgaaaacccactgccccctgagagccgccgtgaccccagccgccggagtgtgcgccagagagaagcctcagggcagcgtggccgctcccgaggaagaggacaccgaccccagacgcctggtgcagctgctgcggcagcacagcagcccttggcaggtgtacggcttcgtgcgggcctgcctgagaaggctggtgccccctggcctgtggggcagcaggcacaacgagcggcggtttctgcggaacaccaagaagttcatcagcctggggaagcacgccaagctgtccctgcaggaactgacctggaagatgagcgtgcggggctgcgcctggctgagaagatcccctggcgtgggctgcgtgcctgccgccgagcaccggctgcgggaggaaatcctggccaagttcctgcactggctgatgagcgtgtacgtggtggagctgctgagatccttcttctacgtgaccgagaccaccttccagaagaactacctgttcttctaccggaagagcgtgtggagcaagctgcagagcatcggcatccggcagcacctgaagcgggtgcagctgagagagctgtccgaggccgaagtgaggcagcaccgggaggccagacctgccctgctgaccagccggctgcggttcatccccaagcccgacggcctgcggcccatcgtgaacatggactacgtggtgggcgccaggaccttccggcgggagaagcgggccgagcggctgacctcgagggtgaaggccctgttcagcgtgctgaactacgagcgggccaggcggccaggcctgctgggcgccagcgtgctgggcctggacgacatccaccgggcctggcggaccttcgtgctgagagtgcgggcccaggacccccctcccgagctgtacttcgtgaaggtggacgtgacaggcgcctacgacaccatcccccaggaccggctgaccgaggtgatcgccagcatcatcaagccccagaacacctactgcgtgcggagatacgccgtggtgcagaaggccgcccacggccacgtgcggaaggccttcaagagccacgtgagcaccctgaccgacctgcagccctacatgcggcagttcgtggcccacctgcaggaaaccagccccctgcgggatgccgtggtgatcgagcagagcagcagcctgaacgaggccagcagcggcctgttcgacgtgttcctgagattcatgtgccaccacgccgtgcggatccggggcaagagctacgtgcagtgccagggcatcccacagggcagcatcctgtccaccctgctgtgctccctgtgctacggcgacatggaaaacaagctgttcgccggcatcaggcgggacggactgctgctgagactggtggacgacttcctgctggtgaccccccacctgacccacgccaagacctttctgcggaccctggtgcgcggcgtgcccgagtacggctgcgtggtgaacctgagaaagaccgtggtgaacttccccgtggaggacgaggccctgggcggcacagccttcgtgcagatgcctgcccatggactgttcccttggtgcgggctgctgctggacacccggaccctggaagtgcagagcgactacagcagctacgcccggaccagcatccgggcctccctgaccttcaacaggggcttcaaggccggcaggaacatgcggcggaagctgtttggcgtgctgcggctgaagtgccacagcctgtttctgtacctgcaggtgaacagcctgcagaccgtgtgcaccaacatctacaagatcctgctgctgcaggcctaccggttccacgcctgcgtgctgcagctgccctttcaccagcaggtgtggaagaaccctaccttcttcctgcgggtgatcagcgacaccgccagcctgtgctacagcatcctgaaggccaagaacgccggcatgagcctgggcgccaagggagccgccggacctctgcccagcgaggccgtgcagtggctgtgccaccaggcctttctgctgaagctgacccggcaccgggtgacctacgtgcccctgctgggcagcctgcggaccgcccagacccagctgtcccggaagctgcctggcaccaccctgacagccctggaagccgccgccaaccccgccctgccctccgacttcaagaccatcctggactacccctacgacgtgcccgactacgcctgatgagcggccgcgagctc

SEQ ID NO: 35 - protein, 1158 aa, Homo sapiens
MDWTWILFLVAAATRVHSPRAPRCRAVRSLLRSHYREVLPLATFVRRLGPQGWRLVQRGDPAAFRALVAQCLVCVPWDARPPPAAPSFRQVSCLKELVARVLQRLCERGAKNVLAFGFALLDGARGGPPEAFTTSVRSYLPNTVTDALRGSGAWGLLLRRVGDDVLVHLLARCALFVLVAPSCAYQVCGPPLYQLGAATQARPPPHASGPRRRLGCERAWNHSVREAGVPLGLPAPGARRRGGSASRSLPLPKRPRRGAAPEPERTPVGQGSWAHPGRTRGPSDRGFCVVSPARPAEEATSLEGALSGTRHSHPSVGRQHHAGPPSTSRPPRPWDTPCPPVYAETKHFLYSSGDKEQLRPSFLLSSLRPSLTGARRLVETIFLGSRPWMPGTPRRLPRLPQRYWQMRPLFLELLGNHAQCPYGVLLKTHCPLRAAVTPAAGVCAREKPQGSVAAPEEEDTDPRRLVQLLRQHSSPWQVYGFVRACLRRLVPPGLWGSRHNERRFLRNTKKFISLGKHAKLSLQELTWKMSVRGCAWLRRSPGVGCVPAAEHRLREEILAKFLHWLMSVYVVELLRSFFYVTETTFQKNYLFFYRKSVWSKLQSIGIRQHLKRVQLRELSEAEVRQHREARPALLTSRLRFIPKPDGLRPIVNMDYVVGARTFRREKRAERLTSRVKALFSVLNYERARRPGLLGASVLGLDDIHRAWRTFVLRVRAQDPPPELYFVKVDVTGAYDTIPQDRLTEVIASIIKPQNTYCVRRYAVVQKAAHGHVRKAFKSHVSTLTDLQPYMRQFVAHLQETSPLRDAVVIEQSSSLNEASSGLFDVFLRFMCHHAVRIRGKSYVQCQGIPQGSILSTLLCSLCYGDMENKLFAGIRRDGLLLRLVDDFLLVTPHLTHAKTFLRTLVRGVPEYGCVVNLRKTVVNFPVEDEALGGTAFVQMPAHGLFPWCGLLLDTRTLEVQSDYSSYARTSIRASLTFNRGFKAGRNMRRKLFGVLRLKCHSLFLYLQVNSLQTVCTNIYKILLLQAYRFHACVLQLPFHQQVWKNPTFFLRVISDTASLCYSILKAKNAGMSLGAKGAAGPLPSEAVQWLCHQAFLLKLTRHRVTYVPLLGSLRTAQTQLSRKLPGTTLTALEAAANPALPSDFKTILDYPYDVPDYA

SEQ ID NO: 36 - DNA, 1707 bp, Artificial Sequence
  Influenza H5N1 HA consensus sequence
atggaaaagatcgtgctgctgttcgccatcgtgagcctggtgaagagcgaccagatctgcatcggctaccacgccaacaacagcaccgagcaggtggacaccatcatggaaaaaaacgtgaccgtgacccacgcccaggacatcctggaaaagacccacaacggcaagctgtgcgacctggacggcgtgaagcccctgatcctgcgggactgcagcgtggccggctggctgctgggcaaccccatgtgcgacgagttcatcaacgtgcccgagtggagctacatcgtggagaaggccaaccccgtgaacgacctgtgctaccccggcgacttcaacgactacgaggaactgaagcacctgctgtcccggatcaaccacttcgagaagatccagatcatccccaagagcagctggtccagccacgaggccagcctgggcgtgagcagcgcctgcccataccagggcaagtccagcttcttccggaacgtggtgtggctgatcaagaagaacagcacctaccccaccatcaagcggagctacaacaacaccaaccaggaagatctgctggtcctgtggggcatccaccaccccaacgacgccgccgagcagaccaagctgtaccagaaccccaccacctacatcagcgtgggcaccagcaccctgaaccagcggctggtgccccggatcgccacccggtccaaggtgaacggccagagcggccggatggaattcttctggaccatcctgaagcccaacgatgccatcaacttcgagagcaacggcaacttcatcgcccccgagtacgcctacaagatcgtgaagaagggcgacagcaccatcatgaagagcgagctggaatacggcaactgcaacaccaagtgccagacccccatgggcgccatcaacagcagcatgcccttccacaacatccaccccctgaccatcggcgagtgccccaagtacgtgaagagcaacaggctggtgctggccaccggcctgcggaacagcccccagcgggagcggcgggccgccgcccggggcctgttcggcgccatcgccggcttcatcgagggcggctggcagggcatggtggacgggtggtacggctaccaccacagcaatgagcagggcagcggctacgccgccgacaaagagagcacccagaaggccatcgacggcgtcaccaacaaggtgaacagcatcatcgacaagatgaacacccagttcgaggccgtgggccgggagttcaacaacctggaacggcggatcgagaacctgaacaagaaaatggaagatggcttcctggacgtgtggacctacaacgccgagctgctggtgctgatggaaaacgagcggaccctggacttccacgacagcaacgtgaagaacctgtacgacaaagtgcggctgcagctgcgggacaacgccaaagagctgggcaacggctgcttcgagttctaccacaagtgcgacaacgagtgcatggaaagcgtgcggaacggcacctacgactacccccagtacagcgaggaagcccggctgaagcgggaggaaatcagcggcgtgaaactggaaagcatcggcatctaccagatcctgagcatctacagcaccgtggccagcagcctggccctggccatcatggtggccggcctgagcctgtggatgtgcagcaacggcagcctgcagtgccggatctgcatctag

SEQ ID NO: 37 - protein, 568 aa, Artificial Sequence
  Influenza H5N1 HA consensus sequence
MEKIVLLFAIVSLVKSDQICIGYHANNSTEQVDTIMEKNVTVTHAQDILEKTHNGKLCDLDGVKPLILRDCSVAGWLLGNPMCDEFINVPEWSYIVEKANPVNDLCYPGDFNDYEELKHLLSRINHFEKIQIIPKSSWSSHEASLGVSSACPYQGKSSFFRNVVWLIKKNSTYPTIKRSYNNTNQEDLLVLWGIHHPNDAAEQTKLYQNPTTYISVGTSTLNQRLVPRIATRSKVNGQSGRMEFFWTILKPNDAINFESNGNFIAPEYAYKIVKKGDSTIMKSELEYGNCNTKCQTPMGAINSSMPFHNIHPLTIGECPKYVKSNRLVLATGLRNSPQRERRAAARGLFGAIAGFIEGGWQGMVDGWYGYHHSNEQGSGYAADKESTQKAIDGVTNKVNSIIDKMNTQFEAVGREFNNLERRIENLNKKMEDGFLDVWTYNAELLVLMENERTLDFHDSNVKNLYDKVRLQLRDNAKELGNGCFEFYHKCDNECMESVRNGTYDYPQYSEEARLKREEISGVKLESIGIYQILSIYSTVASSLALAIMVAGLSLWMCSNGSLQCRICI

SEQ ID NO: 38 - DNA, 1466 bp, Artificial Sequence
  Influenza H1N1&H5N1 NA consensus Sequence
ggtaccgaattcgccaccatggactggacctggatcctgttcctggtggccgctgccacccgggtgcacagcatgaaccccaaccagaagatcatcaccatcggcagcatctgcatggtgatcggcatcgtgagcctgatgctgcagatcggcaacatgatcagcatctgggtgtcccacagcatccagaccggcaaccagcaccaggccgagcccatcagcaacaccaactttctgaccgagaaggccgtggccagcgtgaccctggccggcaacagcagcctgtgccccatcagcggctgggccgtgtacagcaaggacaacagcatccggatcggcagcaagggcgacgtgttcgtgatccgggagcccttcatcagctgcagccacctggaatgccggaccttcttcctgacccagggggccctgctgaacgacaagcacagcaacggcaccgtgaaggacagaagcccctaccggaccctgatgagctgccccgtgggcgaggcccccagcccctacaacagccggttcgagagcgtggcctggtccgccagcgcctgccacgacggcaccagctggctgaccatcggcatcagcggccctgacaacggcgccgtggccgtgctgaagtacaacggcatcatcaccgacaccatcaagagctggcggaacaacatcctgcggacccaggaaagcgagtgcgcctgcgtgaacggcagctgcttcaccgtgatgaccgacggccccagcaacggccaggccagctacaagatcttcaagatggaaaagggcaaggtggtgaagagcgtggagctggacgcccccaactaccactacgaggaatgcagctgctaccccgacgccggcgagatcacctgcgtgtgccgggacaactggcacggcagcaaccggccctgggtgtccttcaaccagaacctggaataccagatcggctacatctgcagcggcgtgttcggcgacaaccccaggcccaacgatggcaccggcagctgcggccctgtgagcgccaacggcgcctacggcgtgaagggcttcagcttcaagtacggcaacggcgtgtggatcggccggaccaagagcaccaacagcagatccggcttcgagatgatctgggaccccaacggctggaccgagaccgacagcagcttcagcgtgaagcaggacatcgtggccatcaccgactggtccggctacagcggcagcttcgtgcagcaccccgagctgaccggcctggactgcatccggccctgcttttgggtggagctgatcagaggcaggcccaaagagagcaccatctggaccagcggcagcagcatcagcttttgcggcgtgaacagcgacaccgtgagctggtcctggcccgacggcgccgagctgcccttcaccatcgacaagtacccctacgacgtgcccgactacgcctgatgagcggccgcgagctc

SEQ ID NO: 39 - protein, 476 aa, Artificial Sequence
  Influenza H1N1&H5N1 NA consensus sequence
MDWTWILFLVAAATRVHSMNPNQKIITIGSICMVIGIVSLMLQIGNMISIWVSHSIQTGNQHQAEPISNTNFLTEKAVASVTLAGNSSLCPISGWAVYSKDNSIRIGSKGDVFVIREPFISCSHLECRTFFLTQGALLNDKHSNGTVKDRSPYRTLMSCPVGEAPSPYNSRFESVAWSASACHDGTSWLTIGISGPDNGAVAVLKYNGIITDTIKSWRNNILRTQESECACVNGSCFTVMTDGPSNGQASYKIFKMEKGKVVKSVELDAPNYHYEECSCYPDAGEITCVCRDNWHGSNRPWVSFNQNLEYQIGYICSGVFGDNPRPNDGTGSCGPVSANGAYGVKGFSFKYGNGVWIGRTKSTNSRSGFEMIWDPNGWTETDSSFSVKQDIVAITDWSGYSGSFVQHPELTGLDCIRPCFWVELIRGRPKESTIWTSGSSISFCGVNSDTVSWSWPDGAELPFTIDKYPYDVPDYA

SEQ ID NO: 40 - DNA, 875 bp, Artificial Sequence
  Influenza H1N1&H5N1 M1 consensus sequence
ggtaccggatccgccaccatggactggacctggattctgttcctggtggccgctgccacccgggtgcacagcatgagcctgctgaccgaggtggagacctacgtgctgtccatcatccccagcggccctctgaaggccgagatcgcccagcggctggaagatgtgttcgccggcaagaacaccgacctggaagccctgatggaatggctgaaaacccggcccatcctgagccccctgaccaagggcatcctgggcttcgtgttcaccctgaccgtgcccagcgagcggggcctgcagcggcggagattcgtgcagaacgccctgaacggcaacggcgaccccaacaacatggaccgggccgtgaagctgtacaagaagctgaagcgggagatcaccttccacggcgccaaagaggtggccctgagctacagcacaggcgccctggccagctgcatgggcctgatctacaaccggatgggcaccgtgaccaccgaggtggccttcggcctggtgtgcgccacctgcgagcagatcgccgacagccagcacagatcccaccggcagatggccaccaccaccaaccccctgatccggcacgagaaccggatggtcctggcctccaccaccgccaaggccatggaacagatggccggcagcagcgagcaggccgccgaagccatggaagtggccagccaggccaggcagatggtgcaggccatgcggaccatcggcacccaccccagcagcagcgccggactgcgggacgacctgctggaaaacctgcaggcctaccagaaacggatgggcgtgcagatgcagcggttcaagtacccctacgacgtgcccgactacgcctgatgagcggccgcgagctc

SEQ ID NO: 41 - protein, 279 aa, Artificial Sequence
  Influenza H1N1&H5N1 M1 consensus sequence
MDWTWILFLVAAATRVHSMSLLTEVETYVLSIIPSGPLKAEIAQRLEDVFAGKNTDLEALMEWLKTRPILSPLTKGILGFVFTLTVPSERGLQRRRFVQNALNGNGDPNNMDRAVKLYKKLKREITFHGAKEVALSYSTGALASCMGLIYNRMGTVTTEVAFGLVCATCEQIADSQHRSHRQMATTTNPLIRHENRMVLASTTAKAMEQMAGSSEQAAEAMEVASQARQMVQAMRTIGTHPSSSAGLRDDLLENLQAYQKRMGVQMQRFKYPYDVPDYA

SEQ ID NO: 42 - DNA, 1700 bp, Artificial Sequence
  Influenza H5N1 M2E-NP consensus sequence
ggtaccgaattcgccaccatggactggacctggatcctgttcctggtcgctgccgccaccagggtgcacagcagcctgctgaccgaggtggagacccccacccggaacgagtggggctgccggtgcagcgacagcagcgaccggggcaggaagcggagaagcgccagccagggcaccaagcggagctacgagcagatggaaacaggcggcgagcggcagaacgccaccgagatccgggccagcgtgggcagaatggtcggcggcatcggccggttctacatccagatgtgcaccgagctgaagctgtccgactacgagggccggctgatccagaacagcatcaccatcgagcggatggtgctgtccgccttcgacgagcggcggaacagatacctggaagagcaccccagcgccggcaaggaccccaagaaaaccggcggacccatctaccggcggagggacggcaagtgggtgcgggagctgatcctgtacgacaaagaggaaatccggcggatctggcggcaggccaacaacggcgaggacgccacagccggcctgacccacctgatgatctggcacagcaacctgaacgacgccacctaccagcggacaagggctctggtccggaccggcatggacccccggatgtgcagcctgatgcagggcagcacactgcccagaagaagcggagccgctggcgcagccgtgaagggcgtgggcaccatggtgatggaactgatccggatgatcaagcggggcatcaacgaccggaatttttggaggggcgagaacggcaggcggacccggatcgcctacgagcggatgtgcaacatcctgaagggcaagttccagacagccgcccagcgggccatgatggaccaggtccgggagagccggaaccccggcaacgccgagatcgaggacctgatcttcctggccagaagcgccctgatcctgcggggcagcgtggcccacaagagctgcctgcccgcctgcgtgtacggactggccgtggccagcggctacgacttcgagcgggagggctacagcctggtcggcatcgaccccttccggctgctgcagaactcccaggtgttcagcctgatccggcccaacgagaaccccgcccacaagtcccagctggtctggatggcctgccacagcgccgccttcgaggatctgagagtgagcagcttcatccggggcaccagagtggtgcccaggggccagctgtccaccaggggcgtgcagatcgccagcaacgagaacatggaagccatggacagcaacaccctggaactgcggagccggtactgggccatccggaccagaagcggcggcaacaccaaccagcagcgggccagcgccggacagatcagcgtgcagcccaccttctccgtgcagcggaacctgcccttcgagagggccaccatcatggccgccttcaccggcaacaccgagggccggaccagcgacatgcggaccgagatcatcaggatgatggaaagcgccaggcccgaggacgtgagcttccagggcaggggcgtgttcgagctgtccgatgagaaggccaccaaccccatcgtgcccagcttcgacatgaacaacgagggcagctacttcttcggcgacaacgccgaggaatacgacaactacccctacgacgtgcccgactacgcctgatgagcggccgcgagctc

SEQ ID NO: 43 - protein, 554 aa, Artificial Sequence
  Influenza H5N1 M2E-NP consensus sequence
MDWTWILFLVAAATRVHSSLLTEVETPTRNEWGCRCSDSSDRGRKRRSASQGTKRSYEQMETGGERQNATEIRASVGRMVGGIGRFYIQMCTELKLSDYEGRLIQNSITIERMVLSAFDERRNRYLEEHPSAGKDPKKTGGPIYRRRDGKWVRELILYDKEEIRRIWRQANNGEDATAGLTHLMIWHSNLNDATYQRTRALVRTGMDPRMCSLMQGSTLPRRSGAAGAAVKGVGTMVMELIRMIKRGINDRNFWRGENGRRTRIAYERMCNILKGKFQTAAQRAMMDQVRESRNPGNAEIEDLIFLARSALILRGSVAHKSCLPACVYGLAVASGYDFEREGYSLVGIDPFRLLQNSQVFSLIRPNENPAHKSQLVWMACHSAAFEDLRVSSFIRGTRVVPRGQLSTRGVQIASNENMEAMDSNTLELRSRYWAIRTRSGGNTNQQRASAGQISVQPTFSVQRNLPFERATIMAAFTGNTEGRTSDMRTEIIRMMESARPEDVSFQGRGVFELSDEKATNPIVPSFDMNNEGSYFFGDNAEEYDNYPYDVPDYA